European Patent Application EP 4 230 641 A2, published August 23, 2023. Title: HUMAN CD30 LIGAND ANTIGEN BINDING PROTEINS. Applicant: Amgen Inc. The sequence listing filed with the application follows.

SEQUENCE LISTING (75 sequences)

SEQ ID NO: 1 - protein, 14 aa, Homo sapiens
TGTSSDVGVYDYVS

SEQ ID NO: 2 - protein, 14 aa, Homo sapiens
TGTSSDVGLYNYVS

SEQ ID NO: 3 - protein, 14 aa, Homo sapiens
TGTSSDIGLYDYVS

SEQ ID NO: 4 - protein, 14 aa, Homo sapiens
TGTSSDIGLYNYVS

SEQ ID NO: 5 - protein, 14 aa, Homo sapiens
TGSSSDIGTYNYVS

SEQ ID NO: 6 - protein, 14 aa, Homo sapiens
TGTSSDVGLYNYVS

SEQ ID NO: 7 - protein, 7 aa, Homo sapiens
EVSNRPS

SEQ ID NO: 8 - protein, 7 aa, Homo sapiens
EVNNRPS

SEQ ID NO: 9 - protein, 7 aa, Homo sapiens
EVINRPS

SEQ ID NO: 10 - protein, 7 aa, Homo sapiens
EVSKRPS

SEQ ID NO: 11 - protein, 10 aa, Homo sapiens
SSYTSRSTWV

SEQ ID NO: 12 - protein, 10 aa, Homo sapiens
SSYTSSSTWV

SEQ ID NO: 13 - protein, 10 aa, Homo sapiens
SSYSSSSTWV

SEQ ID NO: 14 - protein, 5 aa, Homo sapiens
SYIWS

SEQ ID NO: 15 - protein, 5 aa, Homo sapiens
SYYWT

SEQ ID NO: 16 - protein, 5 aa, Homo sapiens
SYSWS

SEQ ID NO: 17 - protein, 5 aa, Homo sapiens
NNYWS

SEQ ID NO: 18 - protein, 5 aa, Homo sapiens
SYYWS

SEQ ID NO: 19 - protein, 16 aa, Homo sapiens
RIYASGNTNYNPSLKS

SEQ ID NO: 20 - protein, 16 aa, Homo sapiens
RIYASGQTNYNPSLKS

SEQ ID NO: 21 - protein, 16 aa, Homo sapiens
RIYTSGITNYNPSLKS

SEQ ID NO: 22 - protein, 16 aa, Homo sapiens
RTSTSGRNNYNPSLKS

SEQ ID NO: 23 - protein, 16 aa, Homo sapiens
RVYSSGLTNYKPSLKS

SEQ ID NO: 24 - protein, 16 aa, Homo sapiens
RIFASGSTNYNPSLRS

SEQ ID NO: 25 - protein, 16 aa, Homo sapiens
DYRVAGTYYYYYGLDV

SEQ ID NO: 26 - protein, 16 aa, Homo sapiens
ERVVGASRYYYYGVDV

SEQ ID NO: 27 - protein, 16 aa, Homo sapiens
DFTIAARRYYYYGMDV

SEQ ID NO: 28 - protein, 16 aa, Homo sapiens
ERATVTTRYHYDGMDV

SEQ ID NO: 29 - protein, 16 aa, Homo sapiens
ERVGVQDYYHYSGMDV

SEQ ID NO: 30 - protein, 14 aa, synthetic construct
  REGION 1..14: note = CONSENSUS SEQUENCE
  SITE 3: note = MISC_FEATURE - XAA CAN BE THR OR SER
  SITE 7: note = MISC_FEATURE - XAA CAN BE VAL OR ILE
  SITE 9: note = MISC_FEATURE - XAA CAN BE VAL, THR OR LEU
  SITE 11: note = MISC_FEATURE - XAA CAN BE ASP OR ASN
TGXSSDXGXYXYVS

SEQ ID NO: 31 - protein, 7 aa, synthetic construct
  REGION 1..7: note = CONSENSUS SEQUENCE
  SITE 3: note = MISC_FEATURE - XAA CAN BE SER, ASN OR ILE
  SITE 4: note = MISC_FEATURE - XAA CAN BE ASN OR LYS
EVXXRPS

SEQ ID NO: 32 - protein, 10 aa, synthetic construct
  REGION 1..10: note = CONSENSUS SEQUENCE
  SITE 4: note = MISC_FEATURE - XAA CAN BE THR OR SER
  SITE 6: note = MISC_FEATURE - XAA CAN BE ARG OR SER
SSYXSXSTWV

SEQ ID NO: 33 - skipped

SEQ ID NO: 34 - protein, 16 aa, synthetic construct
  REGION 1..16: note = CONSENSUS SEQUENCE
  SITE 2: note = MISC_FEATURE - XAA CAN BE ILE, VAL OR THR
  SITE 3: note = MISC_FEATURE - XAA CAN BE TYR, PHE OR SER
  SITE 4: note = MISC_FEATURE - XAA CAN BE THR, SER OR ALA
  SITE 7: note = MISC_FEATURE - XAA CAN BE ILE, LEU, ASN, SER, ARG OR GLN
  SITE 8: note = MISC_FEATURE - XAA CAN BE THR OR ASN
  SITE 11: note = MISC_FEATURE - XAA CAN BE ASN OR LYS
  SITE 15: note = MISC_FEATURE - XAA CAN BE LYS OR ARG
RXXXSGXXNYXPSLXS

SEQ ID NO: 35 - protein, 16 aa, synthetic construct
  REGION 1..16: note = CONSENSUS SEQUENCE
  SITE 1: note = MISC_FEATURE - XAA CAN BE GLU OR ASP
  SITE 2: note = MISC_FEATURE - XAA CAN BE ARG, THR OR PHE
  SITE 3: note = MISC_FEATURE - XAA CAN BE VAL, ALA, ARG OR THR
  SITE 4: note = MISC_FEATURE - XAA CAN BE VAL, THR, GLY OR ILE
  SITE 5: note = MISC_FEATURE - XAA CAN BE VAL, ALA OR GLY
  SITE 6: note = MISC_FEATURE - XAA CAN BE ALA, THR, GLY OR GLN
  SITE 7: note = MISC_FEATURE - XAA CAN BE THR, ASP, ARG OR SER
  SITE 8: note = MISC_FEATURE - XAA CAN BE ARG OR TYR
  SITE 10: note = MISC_FEATURE - XAA CAN BE THR OR HIS
  SITE 12: note = MISC_FEATURE - XAA CAN BE THR ASP OR SER
  SITE 14: note = MISC_FEATURE - XAA CAN BE MET, LEU OR VAL
XXXXXXXXYXYXGXDV

SEQ ID NO: 36 - protein, 110 aa, Homo sapiens
QSALTQPASVSGSPGQSITISCTGTSSDVGVYDYVSWYQQHPGKAPKLMIYEVSNRPSGVSNRFSGSKSGNTASLTISGLQTEDEADYYCSSYTSRSTWVFGGGTKLTVL

SEQ ID NO: 37 - DNA, 326 bp, Homo sapiens
  source 1..326: mol_type = other DNA
cagtctgccctgactcagcctgcctccgtgtctgggtctcctggacagtcgatcaccatctcctgcactggaaccagcagtgacgttggtgtttatgactatgtctcctggtatcaacagcacccaggcaaagcccccaaactcatgatttatgaggtcagtaatcggccctcaggggtttctaatcgcttctctggctccaagtctggcaacacggcctccctgaccatctctgggctccaaactgaggacgaggctgattattactgcagctcatatacaagcaggagcacttgggtgttcggcggagggaccaagctgaccgt

SEQ ID NO: 38 - protein, 110 aa, Homo sapiens
QSALTQPASVSGSPGQSITISCTGTSSDVGLYNYVSWYQQHPDKAPKLMIFEVNNRPSGVSNRFSGSNSGNTASLTISGLQAEDEADYYCSSYTSSSTWVFGGGTKLTVL

SEQ ID NO: 39 - DNA, 330 bp, Homo sapiens
  source 1..330: mol_type = other DNA
cagtctgccctgactcagcctgcctccgtgtctgggtctcctggacagtcgatcaccatctcctgcactggaaccagcagtgacgttggtctttataactatgtctcctggtaccaacagcacccagacaaagcccccaaactcatgatttttgaggtcaataatcggccctcaggggtttctaatcgcttctctggctccaactctggcaacacggcctccctgaccatctctgggctccaggctgaggacgaggctgattattactgcagctcatatacaagcagcagcacttgggtgttcggcggagggaccaagttgaccgtccta

SEQ ID NO: 40 - protein, 110 aa, Homo sapiens
QSALTQPASVSGSPGQSITISCTGTSSDIGLYDYVSWYQQHPDRAPKLIIFEVNNRPSGVSYRFSGSNSGNTASLTISGLQAEDEADYYCSSYTSSSTWVFGGGTKLTVL

SEQ ID NO: 41 - DNA, 326 bp, Homo sapiens
  source 1..326: mol_type = other DNA
cagtctgccctgactcagcctgcctccgtgtctgggtctcctggacagtcgatcaccatctcctgcactggaaccagcagtgacattggtctttatgactatgtctcctggtaccaacagcacccagacagagcccccaaactcataatttttgaggtcaataatcggccctcaggggtttcttatcgcttctctggctccaactctggcaacacggcctccctgaccatctctgggctccaggctgaggacgaggctgattattactgcagctcatatacaagcagcagcacttgggtgttcggcggagggaccaagttgaccgt

SEQ ID NO: 42 - protein, 110 aa, Homo sapiens
QSALTQPASVSGSPGQSITISCTGTSSDIGLYNYVSWYQQHPGKAPKLIIYEVINRPSGVSNRFSGSESGNTASLTISGLQAEDEANYYCSSYTSSSTWVFGGGTKLTVL

SEQ ID NO: 43 - DNA, 330 bp, Homo sapiens
  source 1..330: mol_type = other DNA
cagtctgccctgactcagcctgcctccgtgtctgggtctcctggacagtcgatcaccatctcctgcactggaaccagcagtgacattggtctttataactatgtctcctggtaccaacagcacccaggcaaagcccccaaactcataatttatgaggtcattaatcggccctcaggggtttctaatcgcttctctggctccgagtctggcaacacggcctccctgaccatctctggactccaggctgaggacgaggctaattattactgcagttcatatacaagcagcagcacttgggtgttcggcggagggaccaagctgaccgtcctg

SEQ ID NO: 44 - protein, 110 aa, Homo sapiens
QSALTQPASVSGSPGQSITISCTGSSSDIGTYNYVSWYQQYPGKAPELMIYEVNNRPSGVSDRFSGSTSGNTASLTISGLQANDEADYYCSSYSSSSTWVFGGGTKLTVL

SEQ ID NO: 45 - DNA, 326 bp, Homo sapiens
  source 1..326: mol_type = other DNA
cagtctgccctgactcagcctgcctccgtgtctgggtctcctggacagtcgatcaccatctcctgcactggaagcagcagtgacattggtacttataactatgtctcctggtaccaacagtacccaggcaaagcccccgaactcatgatttatgaggtcaataatcggccctcaggggtttctgatcgcttctctggctccacgtctggcaatacggcctccctgaccatctctgggctccaggctaacgacgaggctgattattactgcagctcatattcaagcagcagcacttgggtgttcggcggagggactaagctgaccgt

SEQ ID NO: 46 - protein, 110 aa, Homo sapiens
QSALTQPASVSGSPGQSITISCTGTSSDVGLYNYVSWYQQQPGKAPKLMIYEVSKRPSGVSNRFSGSTSGNTASLTISGLQADDEADYSCSSYTSSSTWVFGGGTKLTVL

SEQ ID NO: 47 - DNA, 322 bp, Homo sapiens
  source 1..322: mol_type = other DNA
cagtctgccctgactcagcctgcctccgtgtctgggtctcctggacagtcgatcaccatctcctgcactggaactagcagtgacgttggtctttataactatgtctcctggtaccaacagcagccaggcaaagcccccaaactcatgatttatgaggtcagtaagcggccctcaggagtttctaatcgcttctctggctccacgtctggcaacacggcctccctgaccatctctgggctccaggctgacgacgaggctgattattcctgcagctcatatacaagcagcagcacttgggtcttcggcggagggaccaagctga

SEQ ID NO: 48 - protein, 124 aa, Homo sapiens
QVQLQESGPGLVKPSETLSLTCTVSGGSISSYIWSWIRQPAGKGLEWIGRIYASGNTNYNPSLKSRVTISVDTSKNQFSLKLSSMTAADTAVYYCARDYRVAGTYYYYYGLDVWGQGTTVTVSS

SEQ ID NO: 49 - DNA, 372 bp, Homo sapiens
  source 1..372: mol_type = other DNA
caggtgcagctgcaggagtcgggcccaggactggtgaagccttcggagaccctgtccctcacctgcactgtctctggtggctccatcagtagttacatctggagctggatccggcagcccgccggaaagggactggagtggattgggcgtatctatgccagtgggaacaccaactacaacccctccctcaagagtcgagtcaccatatcagtagacacgtccaagaaccagttctccctgaagctgagctctatgaccgccgcggacacggccgtatattactgtgcgagagattatagggtggctggcacttactactactactacggtttggacgtctggggccaagggaccacggtcaccgtctcctca

SEQ ID NO: 50 - protein, 124 aa, Homo sapiens
QVQLQESGPGLVKPSETLSLTCTVSGGSISSYIWSWIRQPAGKGLEWIGRIYASGNTNYNPSLKSRVTMSVDTSKNQFSLKLSSMTAADTAVYYCARDYRVAGTYYYYYGLDVWGQGTTVTVSS

SEQ ID NO: 51 - DNA, 372 bp, Homo sapiens
  source 1..372: mol_type = other DNA
caggtgcagctgcaggagtcgggcccaggactggtgaagccttcggagaccctgtccctcacctgcactgtctctggtggctccatcagtagttacatctggagctggatccggcagcccgccggaaagggactggagtggattgggcgtatctatgccagtgggaacaccaactacaacccctccctcaagagtcgagtcaccatgtcagtagacacgtccaagaaccagttctccctgaagctgagctctatgaccgccgcggacacggccgtatattactgtgcgagagattatagggtggctggcacttactactactactacggtttggacgtctggggccaagggaccacggtcaccgtctcctca

SEQ ID NO: 52 - protein, 124 aa, Homo sapiens
QVQLQESGPGLVKPSETLSLTCTVSGGSISSYIWSWIRQPAGKGLEWIGRIYASGNTNYNPSLKSRVTMSVDTSKNQFSLKLSSVTAADTAVYYCARDYRVAGTYYYYYGLDVWGQGTTVTVSS

SEQ ID NO: 53 - DNA, 372 bp, Homo sapiens
  source 1..372: mol_type = other DNA
caggtgcagctgcaggagtcgggcccaggactggtgaagccttcggagaccctgtccctcacctgcactgtctctggtggctccatcagtagttacatctggagctggatccggcagcccgccggaaagggactggagtggattgggcgtatctatgccagtgggaacaccaactacaacccctccctcaagagtcgagtcaccatgtcagtagacacgtccaagaaccagttctccctgaagctgagctctgtaaccgccgcggacacggccgtatattactgtgcgagagattatagggtggctggcacttactactactactacggtttggacgtctggggccaagggaccacggtcaccgtctcctca

SEQ ID NO: 54 - protein, 124 aa, Homo sapiens
QVQLQESGPGLVKPSETLSLTCTVSGGSISSYIWSWIRQPAGKGLEWIGRIYASGQTNYNPSLKSRVTMSVDTSKNQFSLKLSSMTAADTAVYYCARDYRVAGTYYYYYGLDVWGQGTTVTVSS

SEQ ID NO: 55 - DNA, 366 bp, Homo sapiens
  source 1..366: mol_type = other DNA
cagctgcaggagtcgggcccaggactggtgaagccttcggagaccctgtccctcacctgcactgtctctggtggctccatcagtagttacatctggagctggatccggcagcccgccggaaagggactggagtggattgggcgtatctatgccagtgggcaaaccaactacaacccctccctcaagagtcgagtcaccatgtcagtagacacgtccaagaaccagttctccctgaagctgagctctatgaccgccgcggacacggccgtatattactgtgcgagagattatagggtggctggcacttactactactactacggtttggacgtctggggccaagggaccacggtcaccgtctcctca

SEQ ID NO: 56 - protein, 124 aa, Homo sapiens
QVQLQESGPGLVKPSETLSLTCTVSGGSISSYIWSWIRQPAGKGLEWIGRIYASGQTNYNPSLKSRVTISVDTSKNQFSLKLSSVTAADTAVYYCARDYRVAGTYYYYYGLDVWGQGTTVTVSS

SEQ ID NO: 57 - DNA, 366 bp, Homo sapiens
  source 1..366: mol_type = other DNA
cagctgcaggagtcgggcccaggactggtgaagccttcggagaccctgtccctcacctgcactgtctctggtggctccatcagtagttacatctggagctggatccggcagcccgccggaaagggactggagtggattgggcgtatctatgccagtgggcaaaccaactacaacccctccctcaagagtcgagtcaccatatcagtagacacgtccaagaaccagttctccctgaagctgagctctgtaaccgccgcggacacggccgtatattactgtgcgagagattatagggtggctggcacttactactactactacggtttggacgtctggggccaagggaccacggtcaccgtctcctca

SEQ ID NO: 58 - protein, 124 aa, Homo sapiens
QVQLQESGPGLVKPSETLSLTCTVSGGSISSYIWSWIRQPAGKGLEWIGRIYASGNTNYNPSLKSRVTISVDTSKNQFSLKLSSVTAADTAVYYCARDYRVAGTYYYYYGLDVWGQGTTVTVSS

SEQ ID NO: 59 - DNA, 372 bp, Homo sapiens
  source 1..372: mol_type = other DNA
caggtgcagctgcaggagtcgggcccaggactggtgaagccttcggagaccctgtccctcacctgcactgtctctggtggctccatcagtagttacatctggagctggatccggcagcccgccggaaagggactggagtggattgggcgtatctatgccagtgggaacaccaactacaacccctccctcaagagtcgagtcaccatatcagtagacacgtccaagaaccagttctccctgaagctgagctctgtaaccgccgcggacacggccgtatattactgtgcgagagattatagggtggctggcacttactactactactacggtttggacgtctggggccaagggaccacggtcaccgtctcctca

SEQ ID NO: 60 - protein, 124 aa, Homo sapiens
QVQLQESGPGLVKPSETLSLTCTVSGGSISSYIWSWIRQPAGKGLEWIGRIYASGQTNYNPSLKSRVTISVDTSKNQFSLKLSSMTAADTAVYYCARDYRVAGTYYYYYGLDVWGQGTTVTVSS

SEQ ID NO: 61 - DNA, 379 bp, Homo sapiens
  source 1..379: mol_type = other DNA
cagatgtcaggtgcagctgcaggagtcgggcccaggactggtgaagccttcggagaccctgtccctcacctgcactgtctctggtggctccatcagtagttacatctggagctggatccggcagcccgccggaaagggactggagtggattgggcgtatctatgccagtgggcaaaccaactacaacccctccctcaagagtcgagtcaccatatcagtagacacgtccaagaaccagttctccctgaagctgagctctatgaccgccgcggacacggccgtatattactgtgcgagagattatagggtggctggcacttactactactactacggtttggacgtctggggccaagggaccacggtcaccgtctcctca

SEQ ID NO: 62 - protein, 124 aa, Homo sapiens
QVQLQESGPGLVKPSETLSLTCTVSGGSISSYIWSWIRQPAGKGLEWIGRIYASGQTNYNPSLKSRVTMSVDTSKNQFSLKLSSVTAADTAVYYCARDYRVAGTYYYYYGLDVWGQGTTVTVSS

SEQ ID NO: 63 - DNA, 379 bp, Homo sapiens
  source 1..379: mol_type = other DNA
cagatgtcaggtgcagctgcaggagtcgggcccaggactggtgaagccttcggagaccctgtccctcacctgcactgtctctggtggctccatcagtagttacatctggagctggatccggcagcccgccggaaagggactggagtggattgggcgtatctatgccagtgggcaaaccaactacaacccctccctcaagagtcgagtcaccatgtcagtagacacgtccaagaaccagttctccctgaagctgagctctgtaaccgccgcggacacggccgtatattactgtgcgagagattatagggtggctggcacttactactactactacggtttggacgtctggggccaagggaccacggtcaccgtctcctca

SEQ ID NO: 64 - protein, 124 aa, Homo sapiens
QVQLQESGPGLVKPSETLSLTCTVSGGSISSYYWTWIRQPAGKGLEWIGRIYTSGITNYNPSLKSRVTMSVDTSKNQFSLKLSSVTAADTAVYYCARERVVGASRYYYYGVDVWGQGTTVTVSS

SEQ ID NO: 65 - DNA, 372 bp, Homo sapiens
  source 1..372: mol_type = other DNA
caggtgcagctgcaggagtcgggcccaggactggtgaagccttcggagaccctgtccctcacctgcactgtctctggtggctccatcagtagttactactggacctggatccggcagcccgccgggaagggactggagtggattgggcgtatctataccagtggaatcaccaactacaatccctccctcaagagtcgcgtcaccatgtcagtagacacgtccaagaaccagttctccctgaagctgagctctgtgaccgccgcggacacggccgtgtattactgtgcgagagagcgggtagtgggagctagtaggtactactactacggtgtggacgtctggggccaagggaccacggtcaccgtctcctcc

SEQ ID NO: 66 - protein, 124 aa, Homo sapiens; identical to SEQ ID NO: 64

SEQ ID NO: 67 - DNA, 372 bp, Homo sapiens; identical to SEQ ID NO: 65
  source 1..372: mol_type = other DNA

SEQ ID NO: 68 - protein, 124 aa, Homo sapiens
QVQLQESGPGLVKPSETLSLTCTVSGGSISSYSWSWIRQPAGKGLEWIGRTSTSGRNNYNPSLKSRVTMSVDTSKNQFSLKLNSVTAADTAVYYCARDFTIAARRYYYYGMDVWGQGTTVTVSS

SEQ ID NO: 69 - DNA, 372 bp, Homo sapiens
  source 1..372: mol_type = other DNA
caggtgcagttgcaggagtcgggcccaggactggtgaagccttcggagaccctgtccctcacctgcactgtctctggtggctccatcagtagttactcctggagctggatccggcagcccgccgggaagggactggagtggattgggcgtaccagtaccagtgggagaaacaactacaacccctccctcaagagtcgagtcaccatgtcagttgacacgtccaagaaccagttctccctgaagctgaactctgtgaccgccgcggacacggccgtgtattactgtgcgagagatttcactatagcagctcgtcgctactactactacggtatggacgtctggggccaagggaccacggtcaccgtctcctca

SEQ ID NO: 70 - protein, 124 aa, Homo sapiens
QVQLQESGPRLVKPSETLSLTCTVSGGSITNNYWSWIRQPAGKGLEWIGRVYSSGLTNYKPSLKSRVTMSVDTSKNQFSLRLNSVTAADTAVYYCARERATVTTRYHYDGMDVWGQGTSVTVSS

SEQ ID NO: 71 - DNA, 372 bp, Homo sapiens
  source 1..372: mol_type = other DNA
caggtgcagctgcaggagtcgggcccaagactggtgaagccttcggagaccctgtccctcacctgcactgtctctggtggctccatcactaataactactggagctggatccggcagcccgccgggaaggggctggagtggattgggcgtgtctatagtagtggactcaccaactacaagccctccctcaagagtcgagtcaccatgtcagtagacacgtccaagaaccaattctccctgaggttgaactctgtgaccgccgcggacacggccgtgtattactgtgcgagagagagggcaacagtaactacgaggtaccactacgacggtatggacgtctggggccaagggacctcggtcaccgtctcctca

SEQ ID NO: 72 - protein, 124 aa, Homo sapiens
QVQLQESGPGLVKPSETLSLTCTVSGGSISSYYWSWIRQPAGKGLEWIGRIFASGSTNYNPSLRSRVTMSRDTSKNQFSLKLSSVTAADTAVYYCAKERVGVQDYYHYSGMDVWGQGTTVTVSS

SEQ ID NO: 73 - DNA, 372 bp, Homo sapiens
  source 1..372: mol_type = other DNA
caggtgcagctgcaggagtcgggcccaggactggtgaagccttcggagaccctgtccctcacttgcactgtctctggtggctccatcagtagttactactggagctggatccggcagcccgccgggaagggactggagtggattgggcgcatctttgccagtgggagcaccaactacaacccctccctcaggagtcgagtcaccatgtcaagagacacgtccaagaaccagttctccctgaagctgagttctgtgaccgccgcggacacggccgtttattactgtgcgaaagaaagggtgggagtacaggattactaccactattccggtatggacgtctggggccaagggaccacggtcaccgtctcctca

SEQ ID NO: 74 - protein, 234 aa, Homo sapiens
  REGION 1..37: note = MISC_FEATURE - Cytoplasmic
  REGION 38..62: note = MISC_FEATURE - Transmembrane
  REGION 63..234: note = MISC_FEATURE - Extracellular
MDPGLQQALNGMAPPGDTAMHVPAGSVASHLGTTSRSYFYLTTATLALCLVFTVATIMVLVVQRTDSIPNSPDNVPLKGGNCSEDLLCILKRAPFKKSWAYLQVAKHLNKTKLSWNKDGILHGVRYQDGNLVIQFPGLYFIICQLQFLVQCPNNSVDLKLELLINKHIKKQALVTVCESGMQTKHVYQNLSQFLLDYLQVNTTISVNVDTFQYIDTSTFPLENVLSIFLYSNSD

SEQ ID NO: 75 - skipped